European Patent Specification EP 4 092 041 B1, published August 30, 2023. Title: Novel WhiB family transcriptional regulator WhcA variant and a method for producing L-valine using the same. Applicant: CJ CheilJedang Corporation. The sequence listing filed with the application follows.

SEQUENCE LISTING (10 sequences)

SEQ ID NO: 1 - protein, 116 aa, Artificial Sequence
  WhiB family transcriptional regulator WhcA variant
MTSVIPEQRNNPFYRDSATIASSDHTERGEWVTQAKCRNDDPDALFVRGAAQRRAAAICRHCPVAMQCCADALDNKVEFGVWGGLTERQRRALLRKKPHITNWAEYLAQGGEIAGV

SEQ ID NO: 2 - DNA, 351 bp, Artificial Sequence
  WhiB family transcriptional regulator WhcA variant coding gene
atgacgtctgtgattccagagcagcgcaacaaccccttttatagggacagcgccacaattgcttcctcggaccacacagagcgtggtgagtgggtcactcaggcaaagtgtcgaaatgacgacccagatgcattgtttgttcgtggtgcagcgcaacgccgagcagcagcaatttgccgccactgccctgtagccatgcagtgctgcgccgatgccttagataacaaggtggaattcggagtctggggaggcctgaccgagcgccagcgccgtgcattgcttcgaaagaagccgcacattactaactgggctgaatatttggctcaggggggcgagatcgccggggtttaa

SEQ ID NO: 3 - protein, 116 aa, Artificial Sequence
  Wild-type WhiB family transcriptional regulator WhcA
MTSVIPEQRNNPFYRDSATIASSDHTERGEWVTQAKCRNGDPDALFVRGAAQRRAAAICRHCPVAMQCCADALDNKVEFGVWGGLTERQRRALLRKKPHITNWAEYLAQGGEIAGV

SEQ ID NO: 4 - DNA, 351 bp, Artificial Sequence
  Wild-type WhiB family transcriptional regulator WhcA coding gene
atgacgtctgtgattccagagcagcgcaacaaccccttttatagggacagcgccacaattgcttcctcggaccacacagagcgtggtgagtgggtcactcaggcaaagtgtcgaaatggcgacccagatgcattgtttgttcgtggtgcagcgcaacgccgagcagcagcaatttgccgccactgccctgtagccatgcagtgctgcgccgatgccttagataacaaggtggaattcggagtctggggaggcctgaccgagcgccagcgccgtgcattgcttcgaaagaagccgcacattactaactgggctgaatatttggctcaggggggcgagatcgccggggtttaa

SEQ ID NO: 5 - DNA, 40 bp, Artificial Sequence
  whcA_1F
tgaattcgagctcggtaccctattcgcaactgtgcttacg

SEQ ID NO: 6 - DNA, 33 bp, Artificial Sequence
  whcA_2R
caatgcatctgggtcgtcatttcgacactttgc

SEQ ID NO: 7 - DNA, 33 bp, Artificial Sequence
  whcA_3F
gcaaagtgtcgaaatgacgacccagatgcattg

SEQ ID NO: 8 - DNA, 40 bp, Artificial Sequence
  whcA_4R
gtcgactctagaggatccccatctgcttagttgcatgcgt

SEQ ID NO: 9 - DNA, 20 bp, Artificial Sequence
  whcA_5F
tattcgcaactgtgcttacg

SEQ ID NO: 10 - DNA, 20 bp, Artificial Sequence
  whcA_6R
atctgcttagttgcatgcgt